European Patent Application EP 4 257 679 A1, published October 11, 2023. Title: Cytochrome P450 Enzyme Mutant and Application thereof. Applicant: ASYMCHEM LIFE SCIENCE(TIANJIN)CO.,LTD. The sequence listing filed with the application follows.

SEQUENCE LISTING (1 sequence)

SEQ ID NO: 1 - protein, 1051 aa, P450 enzyme(Bacillus megaterium)
MTIKEMPQPKTFGELKNLPLLNTDKPVQALMKIADELGEIFKFEAPGRVTRYLSSQRLIKEACDESRFDKNLSQALKFVRDFAGDGLFTSWTHEKNWKKAHNILLPSFSQQAMKGYHAMMVDIAVQLVQKWERLNADEHIEVPEDMTRLTLDTIGLCGFNYRFNSFYRDQPHPFITSMVRALDEAMNKLQRANPDDPAYDENKRQFQEDIKVMNDLVDKIIADRKASGEQSDDLLTHMLNGKDPETGEPLDDENIRYQIITFLIAGHETTSGLLSFALYFLVKNPHVLQKAAEEAARVLVDPVPSYKQVKQLKYVGMVLNEALRLWPTAPAFSLYAKEDTVLGGEYPLEKGDELMVLIPQLHRDKTIWGDDVEEFRPERFENPSAIPQHAFKPFGNGQRACIGQQFALHEATLVLGMMLKHFDFEDHTNYELDIKETLTLKPEGFVVKAKSKKIPLGGIPSPSTEQSAKKVRKKAENAHNTPLLVLYGSNMGTAEGTARDLADIAMSKGFAPQVATLDSHAGNLPREGAVLIVTASYNGHPPDNAKQFVDWLDQASADEVKGVRYSVFGCGDKNWATTYQKVPAFIDETLAAKGAENIADRGEADASDDFEGTYEEWREHMWSDVAAYFNLDIENSEDNKSTLSLQFVDSAADMPLAKMHGAFSTNVVASKELQQPGSARSTRHLEIELPKEASYQEGDHLGVIPRNYEGIVNRVTARFGLDASQQIRLEAEEEKLAHLPLAKTVSVEELLQYVELQDPVTRTQLRAMAAKTVCPPHKVELEALLEKQAYKEQVLAKRLTMLELLEKYPACEMKFSEFIALLPSIRPRYYSISSSPRVDEKQASITVSVVSGEAWSGYGEYKGIASNYLAELQEGDTITCFISTPQSEFTLPKDPETPLIMVGPGTGVAPFRGFVQARKQLKEQGQSLGEAHLYFGCRSPHEDYLYQEELENAQSEGIITLHTAFSRMPNQPKTYVQHVMEQDGKKLIELLDQGAHFYICGDGSQMAPAVEATLMKSYADVHQVSEADARLWLQQLEEKGRYAKDVWAGLE